European Patent Specification EP 3 049 113 B1, published December 27, 2023. Title: BINDING MOIETIES FOR BIOFILM REMEDIATION. Applicant: Trellis Bioscience, Inc. Kauvar, Lawerence M. Application Not Yet Assigned. The sequence listing filed with the application follows.

SEQUENCE LISTING (51 sequences)

SEQ ID NO: 1 - protein, 123 aa, Homo sapiens
QVQLVESGGGLVQPGGSLRLSCAASGFPFSSYAMSWVRQAPGKGLEWVSAISGNGADSYYADSVKGRFTTSRDKSKNTVYLQMNRLRAEDTAVYYCAKDMRRYHYDSSGLHFWGQGTLVTVSS

SEQ ID NO: 2 - protein, 109 aa, Homo sapiens
DIELTQAPSVSVYPGQTARITCSGDALPKQYAYWYQQKPGQAPVVVIYKDSERPSGISERFSGSSSGTTVTLTISGVQAGDEADYYCQSVDTSVSYYVVFGGGTKLTVL

SEQ ID NO: 3 - protein, 123 aa, Homo sapiens; identical to SEQ ID NO: 1

SEQ ID NO: 4 - protein, 110 aa, Homo sapiens
DIMLTQPPSVSAAPGQKVTISCSGSSSNIGTNYVSWFQQVPGTAPKFLIYDNYKRPSETPDRFSGSKSGTSATLDITGLQTGDEANYYCATWDSSLSAWVFGGGTKVTVL

SEQ ID NO: 5 - protein, 119 aa, Homo sapiens
QVQLVESGPGLVKPSETLSLTCRVSGDSNRPSYWSWIRQAPGKAMEWIGYVYDSGVTIYNPSLKGRVTISLDTSKTRFSLKLTSVIAADTAVYYCARERFDRTSYKSWWGQGTQVTVSS

SEQ ID NO: 6 - protein, 108 aa, Homo sapiens
DIVLTQAPGTLSLSPGDRATLSCRASQRLGGTSLAWYQHRSGQAPRLILYGTSNRATDTPDRFSGSGSGTDFVLTISSLEPEDFAVYYCQQYGSPPYTFGQGTTLDIK

SEQ ID NO: 7 - protein, 122 aa, Homo sapiens
QVQLVQSGGTLVQPGGSLRLSCAASGFTFSYYSMSWVRQAPGKGLEWVANIKHDGTERNYVDSVKGRFTISRDNSEKSLYLQMNSLRAEDTAVYYCAKYYYGAGTNYPLKYWGQGTRVTVSS

SEQ ID NO: 8 - protein, 108 aa, Homo sapiens
DILMTQSPSSLSASVGDRVTITCRASQGIRNDLGWYQQKPGKAPKLLIYAASSLQSGVPSRFSGSGSGTDFTLTISSLQPEDFATYYCLQDYNYPLTFGGGTKVEIKR

SEQ ID NO: 9 - protein, 116 aa, Homo sapiens
QVQLLESGPGLVRPSDTLSLTCTFSADLSTNAYWTWIRQPPGKGLEWIGYMSHSGGRDYNPSFNRRVTISVDTSKNQVFLRLTSVTSADTAVYFCVREVGSYYDYWGQGILVTVSS

SEQ ID NO: 10 - protein, 108 aa, Homo sapiens
DIEMTQSPSSLSASVGDRITITCRASQGISTWLAWYQQKPGKAPKSLIFSTSSLHSGVPSKFSGSGSGTDFTLTITNLQPEDFATYYCQQKWETPYSFGQGTKLDMIR

SEQ ID NO: 11 - protein, 116 aa, Homo sapiens
QVQLVESGTEVKNPGASVKVSCTASGYKFDEYGVSWVRQSPGQGLEWMGWISVYNGKTNYSQNFQGRLTLTTETSTDTAYMELTSLRPDDTAVYYCATDKNWFDPWGPGTLVTVSS

SEQ ID NO: 12 - protein, 107 aa, Homo sapiens
DIVMTQSPSASGSPGQSITISCTGTNTDYNYVSWYQHHPGKAPKVIIYDVKKRPSGVPSRFSGSRSGNTATLTVSGLQTEDEADYYCVSYADNNHYVFGSGTKVTVL

SEQ ID NO: 13 - protein, 128 aa, Homo sapiens
QVQLVESGGGVVQPGGSLRVSCAASAFSFRDYGIHWVRQAPGKGLQWVAVISHDGGKKFYADSVRGRFTISRDNSENTLYLQMNSLRSDDTAVYYCARLVASCSGSTCTTQPAAFDIWGPGTLVTVSS

SEQ ID NO: 14 - protein, 108 aa, Homo sapiens
DIMLTQPPSVSVSPGQTARITCSGDALPKKYTYWYQQKSGQAPVLLIYEDRKRPSEIPERFSAFTSWTTATLTITGAQVRDEADYYCYSTDISGDIGVFGGGTKLTVL

SEQ ID NO: 15 - protein, 120 aa, Homo sapiens
QVQLLESGADMVQPGRSLRLSCAASGFNFRTYAMHWVRQAPGKGLEWVAVMSHDGYTKYYSDSVRGQFTISRDNSKNTLYLQMNNLRPDDTAIYYCARGLTGLSVGFDYWGQGTLVTVSS

SEQ ID NO: 16 - protein, 111 aa, Homo sapiens
DIVLTQSASVSGSPGQSITISCTGTSSDVGGYNYVSWYQQHPGKAPKLMIYDVTTRPSGVSDRFSGSKSGNTASLTISGLQAEDEADYYCSSYSSGSTPALFGGGTQLTVL

SEQ ID NO: 17 - protein, 122 aa, Homo sapiens
QVQLVQSGGGLVKPGGSLRLSCGASGFNLSSYSMNWVRQAPGKGLEWVSSISSRSSYIYYADSVQGRFTISRDNAKNSLYLQMNSLRAEDTAIYYCARVSPSTYYYYGMDVWGQGTTVTVSS

SEQ ID NO: 18 - protein, 108 aa, Homo sapiens
DIVLTQPSSVSVSPGQTARITCSGDELPKQYAYWYQQKPGQAPVLVIYKDNERPSGIPERFSGSSSGTTVTLTISGVQAEDEADYYCQSADSSGTYVVFGGGTKLTVL

SEQ ID NO: 19 - protein, 136 aa, Homo sapiens
QVQLVESGAEVKKPGALVKVSCKASGYTFSGYYMHWVRQAPGQGLEWMGWINPKSGGTKYAQKFQGRVTMTRDTSISTAYMELSRLRSDDTAVYFCARGGPSNLERFLERLQPRYSYDDKYAMDVWGQGTTVTVSS

SEQ ID NO: 20 - protein, 109 aa, Homo sapiens
DIVMTQSPGTLSLSPGARATLSCRASQSVSSIYLAWYQQKPGQAPRLLIFGASSRATGIPDRFSGSGSGTDFTLTISRLEPEDFAVYYCQQYGSSPYTFGQGTKLEIKR

SEQ ID NO: 21 - protein, 124 aa, Homo sapiens
QVQLVQSGTEVKKPGESLKISCEGSRYNFARYWIGWVRQMPGKGLDWMGIIYPGDSDTRYSPSFQGQVSISADKSISTAYLQWNSLKASDTAMYYCARLGSELGVVSDYYFDSWGQGTLVTVSS

SEQ ID NO: 22 - protein, 114 aa, Homo sapiens
DIVLTQSPDSLAVSLGERATINCKSSQSVLDRSNNKNCVAWYQQKPGQPPKLLIYRAATRESGVPDRFSGSGSGTDFSLTISSLQAEDVAVYFCQQYYSIPNTFGQGTKLEIKR

SEQ ID NO: 23 - protein, 120 aa, Homo sapiens
QVQLVESGGGLVKAGGSLRLSCVASGFTFSDYYMSWIRQAPGKGLEWISFISSSGDTIFYADSVKGRFTVSRDSAKNSLYLQMNSLKVEDTAVYYCARKGVSDEELLRFWGQGTLVTVSS

SEQ ID NO: 24 - protein, 108 aa, Homo sapiens
DIVLTQDPSVSVSPGQTARITCSGDALPKKYAYWYQQKSGQAPVLVIYEDTKRPSGIPERFSGSSSGTVATLTISGAQVEDEADYYCYSTDSSGNQRVFGGGTKLTVL

SEQ ID NO: 25 - DNA, 384 bp, Homo sapiens
caggtgcagctggtgcagtctgggggaggcttggtacagcctggggggtccctgagactctcctgtgcagcctctggatttaccttcagtgattatagtatgaactgggtccgccaggctccagggaagggactggaatggctttcatacattagtcacactattactaccatatactacgccgactctgtgaagggccgattcaccatctccagagacaatgccgacagctcactgtatctccaaatgaacagcctgggagacgaggacacggctgtgtattactgtgcgagagctccattagtaaactgtagtactagtggctgccagtccggaagctggttcgacacctggggccagggaaccctggtcaccgtctcctca

SEQ ID NO: 26 - DNA, 327 bp, Homo sapiens
gatatcgagctgactcaggcaccctcggtgtcagtgtatccaggacagacggccaggatcacctgctctggagatgcactgccaaagcaatatgcttattggtaccagcagaagccaggccaggcccctgtggtggtgatatataaagacagtgagaggccctcagggatctctgagcgattctctggctccagctcggggacaacagtcacgttgaccatcagtggagtccaggcaggggacgaggctgactattattgtcaatcagttgacaccagtgtttcttattatgtggtcttcggcggagggaccaagttgaccgtccta

SEQ ID NO: 27 - DNA, 369 bp, Homo sapiens
caggtgcagctggtggagtccgggggaggcttggtacagcctggggggtccctgagactttcctgtgccgcctctggattccccttcagtagttatgccatgagttgggtccgtcaggctccagggaaggggctggagtgggtctcagccatcagtggcaacggcgctgactcatattacgcagactccgtgaagggccgcttcaccacttccagagacaagtccaagaatacagtttatttgcaaatgaacagactcagggccgaggacacggccgtatattactgtgcgaaagatatgcgacggtatcattatgacagtagtggtctgcacttctggggccagggaaccctggtcaccgtctcctca

SEQ ID NO: 28 - DNA, 330 bp, Homo sapiens
gatatcatgctgactcagcccccctcagtgtctgcggcccccggacagaaggtcaccatctcctgctctggaagcagctccaacattgggacgaattatgtgtcctggttccagcaggtcccaggaacagcccccaaattcctcatttatgacaattataaacgaccctcagaaactcctgaccgattctctggctccaagtctggcacgtcggccaccctggacatcaccggactccagactggggacgaggccaattattactgcgcaacatgggacagtagcctgagtgcttgggtgttcggcggagggaccaaggtgaccgtcctg

SEQ ID NO: 29 - DNA, 357 bp, Homo sapiens
caggtgcagctggtggagtccggcccaggactggtgaagccttcggagaccctgtccctcacctgcagggtctctggtgactccaatcggccttcctactggagctggatcaggcaggccccagggaaggcaatggagtggataggttatgtctatgacagtggggtcaccatctacaatccctccctcaagggtcgagtcacaatatcactagacacgtcgaagacgcggttctccctgaaactgacctctgtgatcgctgcggacacggccgtatattattgtgcgcgagaacgttttgatcggacatcgtataagagttggtggggccagggaacgcaggtcaccgtctcctca

SEQ ID NO: 30 - DNA, 324 bp, Homo sapiens
gatatcgtgctgactcaggccccaggcactctgtctttgtctccaggggacagagccaccctctcctgtagggccagtcagcgtcttggcggcacgtccttagcctggtaccagcacagatctggccaggctcccaggctcatcctctacggaacttcaaacagggccactgacacccctgacaggtttagtggcagtgggtctgggacagacttcgttctcaccatcagttccctggagcctgaagattttgcagtgtattactgtcagcaatatggcagcccaccgtacacttttggccaggggaccactctggacatcaaa

SEQ ID NO: 31 - DNA, 366 bp, Homo sapiens
caggtgcagctggtgcagtctgggggaaccttggtccagccgggggggtccctgagactctcctgtgcagcctctggattcacctttagttactactcgatgagctgggtccgccaggctccagggaaggggctggagtgggtggccaacataaagcacgatggaactgagagaaattatgtggactctgtgaagggccgattcaccatctccagagacaacagcgagaagtctctttacctgcaaatgaacagcctgagagccgaggacacggctgtgtattactgtgcgaagtattattatggtgccgggactaattatccccttaagtactggggccagggaacccgggtcaccgtctcctca

SEQ ID NO: 32 - DNA, 324 bp, Homo sapiens
gatatcctgatgacccagtctccatcctccctgtctgcatctgtaggagacagagtcaccatcacttgccgggcaagtcagggcattagaaatgatttaggctggtatcagcagaaaccagggaaagcccctaagctcctgatctatgctgcatccagtttacaaagtggggtcccatcaaggttcagcggcagtggatctggcacagatttcactctcaccatcagcagcctgcagcctgaagattttgcaacttattactgtctacaagattacaattacccgctcactttcggcggagggaccaaggtggagatcaaacga

SEQ ID NO: 33 - DNA, 348 bp, Homo sapiens
caggtgcagctgctcgagtcaggcccaggcctggttaggccctcggacaccctgtccctcacctgcactttttccgctgacctcagcaccaacgcctattggacctggatccggcagcccccaggaaagggactggagtggattggctatatgtctcatagtgggggaagggattacaatccctccttcaaccggcgagtcaccatttcagtggacacgtcgaagaaccaggttttcttgaggctgacgtcagtgacctctgcggacacggccgtctatttctgtgtgagagaagtcggcagttactacgactactggggccagggaatcctggtcaccgtctcctca

SEQ ID NO: 34 - DNA, 324 bp, Homo sapiens
gatatcgagatgacccagtctccatcctctttgtctgcatctgtcggagacagaatcaccatcacttgtcgggcgagtcagggtattagcacctggttagcctggtatcagcagaaaccggggaaagcccctaagtccctgatcttttctacgtccagcctgcatagtggggtcccctcaaagttcagcggcagtgggtctgggacagacttcactctcaccatcaccaacctgcagcctgaagattttgcaacttattactgccaacagaaatgggagaccccttatagttttggccaggggaccaagctggacatgatacga

SEQ ID NO: 35 - DNA, 348 bp, Homo sapiens
caggtgcagctggtggagtctggaactgaggtgaagaaccctggagcctcagtgaaggtctcctgcacggcctctggttacaaatttgacgaatatggtgtcagttgggtgcgacagtcccctggacaaggacttgagtggatgggatggatcagtgtttataatggcaagacaaactatagccagaactttcagggcagactcaccctgaccacagagacatccaccgacacagcctacatggagcttacgagcctcagacctgacgacacggccgtctattactgtgcgacagacaaaaactggttcgacccctggggcccgggaaccctggtcaccgtctcctca

SEQ ID NO: 36 - DNA, 321 bp, Homo sapiens
gatatcgtgatgacccagtctccctccgcgtccgggtctcctggacagtcaatcaccatctcctgcactggaaccaacactgattataattatgtttcctggtaccagcaccaccccggcaaagcccccaaagtcattatttatgacgtcaaaaagcggccctcgggggtccctagtcgcttctctggctccaggtctggcaacacggccaccctgaccgtctctgggctccagactgaggatgaggctgattattattgtgtctcatatgcagacaacaatcattatgtcttcggaagtgggaccaaggtcaccgtcctg

SEQ ID NO: 37 - DNA, 384 bp, Homo sapiens
caggtgcagctggtggagtccgggggaggcgtggtccagcctggagggtccctgagagtctcctgtgcagcctctgcgttcagtttcagggattatggcatacactgggtccgccaggctccaggcaaggggctgcaatgggtggcggttatttcacatgatggaggtaagaaattctatgcagactccgtgaggggccgattcaccatctccagagacaattccgagaacacactgtatctccaaatgaacagcctgagatctgacgacacggctgtctattactgtgcgaggctcgttgccagttgcagtggttccacctgcacaacgcaacctgctgcctttgacatttggggcccagggacattggtcaccgtctcttca

SEQ ID NO: 38 - DNA, 324 bp, Homo sapiens
gatatcatgctgactcagccgccctcggtgtcagtgtccccaggacaaacggccaggatcacctgctctggagatgcattgccaaaaaaatatacttattggtatcagcagaagtcaggccaggcccctgttctgctcatctatgaggacaggaaacgaccctccgagatccctgagagattctctgccttcacctcatggacgacggccaccttgactatcactggggcccaggtgagagatgaagctgactactactgttattcaacagacatcagtggtgatataggagtgttcggcggagggaccaagctgaccgtccta

SEQ ID NO: 39 - DNA, 333 bp, Homo sapiens
gatatcgtgctgactcagtcggcctccgtgtctgggtctcctggacagtcgatcaccatctcctgcactggaaccagcagtgacgttggtggatataactatgtctcctggtaccaacaacacccaggcaaagcccccaaactcatgatttatgatgtcactactcggccttcaggggtttctgatcgcttctctggctccaagtctggcaacacggcctccctgaccatctctgggctgcaggctgaggacgaggctgattattattgcagctcatattcaagcggctccacacctgctctgtttggggggggcacccagctgaccgtcctc

SEQ ID NO: 40 - DNA, 333 bp, Homo sapiens; identical to SEQ ID NO: 39

SEQ ID NO: 41 - DNA, 366 bp, Homo sapiens
caggtgcagctggtgcagtctgggggaggcctggtcaagcctggggggtccctgagactctcctgtggagcctctggatttaacctcagtagttatagcatgaactgggtccgccaggctccagggaaggggctggagtgggtctcatccattagtagtagaagtagttacatatactatgcagactcagtgcagggccgattcaccatctccagagacaacgccaagaactcactgtatctgcaaatgaacagcctgagagccgaggacacggctatatattactgtgcgagagtatctccgtccacctattattattatggtatggacgtctggggccaagggaccacggtcaccgtctcctca

SEQ ID NO: 42 - DNA, 324 bp, Homo sapiens
gatatcgtactcactcagccgtcctcggtgtcagtgtccccaggacagacggccaggatcacctgctctggagatgaattgccaaagcaatatgcttattggtaccagcagaagccaggccaggcccctgtgttggtaatatataaagacaatgagaggccctcagggatccctgagcgattctctggctccagctcagggacaacagtcacgttgaccatcagtggagtccaggcagaagacgaggctgactattactgtcaatcagcagacagtagtggtacttatgtggtgttcggcggagggaccaagctgaccgtccta

SEQ ID NO: 43 - DNA, 408 bp, Homo sapiens
caggtgcagctggtggagtctggggctgaggtgaagaagcctggggccttagtgaaggtctcctgcaaggcttctggatacaccttcagcggctactatatgcactgggtgcgacaggcccctggacaagggcttgagtggatgggatggatcaaccctaagagtggtggcacaaagtatgcacagaagtttcagggccgggtcaccatgaccagggacacgtccatcagcacagcctacatggagttgagcaggctaagatctgacgacacggccgtgtatttctgtgcgagaggcggaccttcaaatttggaacgatttttggagaggttacaaccccgctacagttacgacgacaagtatgctatggacgtctggggccaagggaccacggtcaccgtctcctca

SEQ ID NO: 44 - DNA, 328 bp, Homo sapiens
gatatcgtgatgacccagtctccaggcaccctgtctttgtctccaggggcaagagccaccctctcctgcagggccagtcagagtgttagcagcatctatttagcctggtaccagcagaaacctggccaggctcccaggctcctcatctttggtgcatccagcagggccactggcatcccagacaggttcagtggcagtgggtctgggacagacttcactctcaccatcagcagactggagcctgaagattttgcagtgtattactgtcagcagtatggtagctcaccgtacacttttggccaggggaccaagctggagatcaaacgaa

SEQ ID NO: 45 - DNA, 372 bp, Homo sapiens
caggtgcagctggtgcagtctggaacagaagtgaaaaagcccggggagtctctgaagatctcctgtgagggttctcgatacaactttgccaggtactggatcggctgggtgcgccagatgcccggaaaaggcctggactggatggggatcatctatcctggtgactccgataccagatacagcccgtccttccaaggccaggtcagcatctcagccgacaagtccatcagtaccgcctacctgcagtggaacagcctgaaggcctcggacaccgccatgtattattgtgcgagacttgggagcgagcttggagtggtctctgattattactttgactcctggggccagggaaccctggtcaccgtctcctca

SEQ ID NO: 46 - DNA, 342 bp, Homo sapiens
gatatcgtgttgactcagtctccagactccctggctgtgtctctgggcgagagggccaccatcaactgcaagtccagccagagtgttttagacaggtccaacaataagaactgtgtagcttggtaccagcagaaaccgggacagcctcctaaactgctcatttaccgggctgctacccgggaatccggggtccctgatcgattcagtggcagcgggtctgggacagacttcagtctcaccatcagcagcctgcaggctgaagatgtggcagtttatttctgtcagcaatattatagtattccgaacacttttggccaggggaccaagctggagatcaaacga

SEQ ID NO: 47 - DNA, 360 bp, Homo sapiens
caggtgcagctggtggagtctgggggaggcttggtcaaggctggagggtccctgagactctcctgtgtagcctctggattcaccttcagcgactactacatgtcctggattcgccaggctccagggaaggggctggagtggatttcatttattagtagtagtggtgataccatattttacgcagactctgtgaagggccgattcaccgtctccagggacagcgccaagaactcactgtatcttcaaatgaacagcctgaaagtcgaggacacggccgtgtattactgtgcgaggaagggggtgtccgacgaggaactactgcgcttctggggccagggaaccctggtcaccgtctcctca

SEQ ID NO: 48 - DNA, 324 bp, Homo sapiens
gatatcgtgctgactcaggacccctcggtgtcagtgtccccaggacaaacggccaggatcacctgctctggagatgcattgccaaaaaaatatgcttattggtaccagcagaagtcaggccaggcccctgtgctggtcatctatgaggacaccaaacgaccctccgggatccctgagagattctctggctccagctcagggacagtggccaccttgactatcagtggggcccaggtggaggatgaagctgactactattgttactcaacagacagcagcggtaatcagagggtattcggcggagggaccaagctgaccgtccta

SEQ ID NO: 49 - protein, 16 aa, H. influenzae
IEYLSDKYHLSKQDTK

SEQ ID NO: 50 - protein, 23 aa, H. influenzae
RDKSSRPGRNPKTGDVVAASARR

SEQ ID NO: 51 - protein, 11 aa, H. influenzae
QKLRARVEKTK